European Patent Application EP 4 574 839 A1, published June 25, 2025. Title: CO-DELIVERY SYSTEM. Applicant: BioNTech SE. The sequence listing filed with the application follows.

SEQUENCE LISTING (25 sequences)

SEQ ID NO: 1 - protein, 107 aa, Homo sapiens
GQPREPQVYTLPPSREEMTKNQVSLTCLVKGFYPSDIAVEWESNGQPENNYKTTPPVLDSDGSFFLYSKLTVDKSRWQQGNVFSCSVMHEALHNHYTQKSLSLSPGK

SEQ ID NO: 2 - protein, 107 aa, synthetic construct
GQPREPQVYTLPPCREEMTKNQVSLWCLVKGFYPSDIAVEWESNGQPENNYKTTPPVLDSDGSFFLYSKLTVDKSRWQQGNVFSCSVMHEALHNHYTQKSLSLSPGK

SEQ ID NO: 3 - protein, 107 aa, synthetic construct
GQPREPQVCTLPPSREEMTKNQVSLSCAVKGFYPSDIAVEWESNGQPENNYKTTPPVLDSDGSFFLVSKLTVDKSRWQQGNVFSCSVMHEALHNHYTQKSLSLSPGK

SEQ ID NO: 4 - protein, 19 aa, synthetic construct
DKTHTCPPCGGGSSGGGSG

SEQ ID NO: 5 - protein, 24 aa, synthetic construct
EPKSCDKTHTCPPCGGGSSGGGSG

SEQ ID NO: 6 - protein, 42 aa, synthetic construct
EPKSCDKTHTCPPCPEPKSCDTPPPCPRCPAPGGGSSGGGSG

SEQ ID NO: 7 - protein, 47 aa, synthetic construct
GGGGSGGGGSDKTHTCPPCPEPKSCDTPPPCPRCPAPGGGSSGGGSG

SEQ ID NO: 8 - protein, 29 aa, synthetic construct
GGGGSGGGGSDKTHTCPPCGGGSSGGGSG

SEQ ID NO: 9 - protein, 29 aa, synthetic construct
GGGGSGGGGSDKTHTSPPSGGGSSGGGSG

SEQ ID NO: 10 - protein, 5 aa, synthetic construct
GGGGS

SEQ ID NO: 11 - protein, 163 aa, synthetic construct
GGGGSGGGGSDKTHTCPPCPEPKSCDTPPPCPRCPAPGGGSSGGGSGGQPREPQVYTLPPCREEMTKNQVSLWCLVKGFYPSDIAVEWESNGQPENNYKTTPPVLDSDGSFFLYSKLTVDKSRWQQGNVFSCSVMHEALHNHYTQKSLSLSPGKGGGGSGGGS

SEQ ID NO: 12 - protein, 154 aa, synthetic construct
GGGGSGGGGSDKTHTCPPCPEPKSCDTPPPCPRCPAPGGGSSGGGSGGQPREPQVCTLPPSREEMTKNQVSLSCAVKGFYPSDIAVEWESNGQPENNYKTTPPVLDSDGSFFLVSKLTVDKSRWQQGNVFSCSVMHEALHNHYTQKSLSLSPGK

SEQ ID NO: 13 - protein, 145 aa, synthetic construct
GGGGSGGGGSDKTHTCPPCGGGSSGGGSGGQPREPQVYTLPPCREEMTKNQVSLWCLVKGFYPSDIAVEWESNGQPENNYKTTPPVLDSDGSFFLYSKLTVDKSRWQQGNVFSCSVMHEALHNHYTQKSLSLSPGKGGGGSGGGS

SEQ ID NO: 14 - protein, 136 aa, synthetic construct
GGGGSGGGGSDKTHTCPPCGGGSSGGGSGGQPREPQVCTLPPSREEMTKNQVSLSCAVKGFYPSDIAVEWESNGQPENNYKTTPPVLDSDGSFFLVSKLTVDKSRWQQGNVFSCSVMHEALHNHYTQKSLSLSPGK

SEQ ID NO: 15 - protein, 145 aa, synthetic construct
GGGGSGGGGSDKTHTSPPSGGGSSGGGSGGQPREPQVYTLPPCREEMTKNQVSLWCLVKGFYPSDIAVEWESNGQPENNYKTTPPVLDSDGSFFLYSKLTVDKSRWQQGNVFSCSVMHEALHNHYTQKSLSLSPGKGGGGSGGGS

SEQ ID NO: 16 - protein, 136 aa, synthetic construct
GGGGSGGGGSDKTHTSPPSGGGSSGGGSGGQPREPQVCTLPPSREEMTKNQVSLSCAVKGFYPSDIAVEWESNGQPENNYKTTPPVLDSDGSFFLVSKLTVDKSRWQQGNVFSCSVMHEALHNHYTQKSLSLSPGK

SEQ ID NO: 17 - protein, 121 aa, synthetic construct
GGGGSGQPREPQVYTLPPCREEMTKNQVSLWCLVKGFYPSDIAVEWESNGQPENNYKTTPPVLDSDGSFFLYSKLTVDKSRWQQGNVFSCSVMHEALHNHYTQKSLSLSPGKGGGGSGGGS

SEQ ID NO: 18 - protein, 112 aa, synthetic construct
GGGGSGQPREPQVCTLPPSREEMTKNQVSLSCAVKGFYPSDIAVEWESNGQPENNYKTTPPVLDSDGSFFLVSKLTVDKSRWQQGNVFSCSVMHEALHNHYTQKSLSLSPGK

SEQ ID NO: 19 - protein, 339 aa, synthetic construct
ASTKGPSVFPLAPSSKSTSGGTAALGCLVKDYFPEPVTVSWNSGALTSGVHTFPAVLQSSGLYSLSSVVTVPSSSLGTQTYICNVNHKPSNTKVDKRVEPKSCDKTHTCPPCPAPELLGGPSVFLFPPKPKDTLMISRTPEVTCVVVDVSHEDPEVKFNWYVDGVEVHNAKTKPREEQYNSTYRVVSVLTVLHQDWLNGKEYKCKVSNKALPAPIEKTISKAKGQPREPQVYTLPPSREEMTKNQVSLTCLVKGFYPSDIAVEWESNGQPENNYKTTPPVLDSDGSFFLYSKLTVDKSRWQQGNVFSCSVMHEALHNHYTQKSLSLSPGKGGGGSGGGS

SEQ ID NO: 20 - protein, 107 aa, synthetic construct [sequence omitted]

SEQ ID NO: 21 - protein, 106 aa, synthetic construct
GQPKANPTVTLFPPSSEELQANKATLVCLISDFYPGAVTVAWKADSSPVKAGVETTTPSKQSNNKYAASSYLSLTPEQWKSHRSYSCQVTHEGSTVEKTVAPTECS

SEQ ID NO: 22 - protein, 107 aa, synthetic construct
GQPREPQVYTLPPSREEMTKNQVSLWCLVKGFYPSDIAVEWESNGQPENNYKTTPPVLDSDGSFFLYSKLTVDKSRWQQGNVFSCSVMHEALHNHYTQKSLSLSPGK

SEQ ID NO: 23 - protein, 107 aa, synthetic construct
GQPREPQVYTLPPSREEMTKNQVSLSCAVKGFYPSDIAVEWESNGQPENNYKTTPPVLDSDGSFFLVSKLTVDKSRWQQGNVFSCSVMHEALHNHYTQKSLSLSPGK

SEQ ID NO: 24 - protein, 107 aa, synthetic construct
GQPREPQVYTLPPCREEMTKNQVSLTCLVKGFYPSDIAVEWESNGQPENNYKTTPPVLDSDGSFFLYSKLTVDKSRWQQGNVFSCSVMHEALHNHYTQKSLSLSPGK

SEQ ID NO: 25 - protein, 107 aa, synthetic construct
GQPREPQVCTLPPSREEMTKNQVSLTCLVKGFYPSDIAVEWESNGQPENNYKTTPPVLDSDGSFFLYSKLTVDKSRWQQGNVFSCSVMHEALHNHYTQKSLSLSPGK